European Patent Specification EP 3 856 775 B9, published January 22, 2025. Title: Chimeric antigen receptor. Applicant: Autolus Limited. The sequence listing filed with the application follows.

SEQUENCE LISTING (88 sequences)

SEQ ID NO: 1 - protein, 106 aa, Artificial Sequence
  kappa chain constant domain
TVAAPSVFIFPPSDEQLKSGTASVVCLLNNFYPREAKVQWKVDNALQSGNSQESVTEQDSKDSTYSLSSTLTLSKADYEKHKVYACEVTHQGLSSPVTKSFNRGEC

SEQ ID NO: 2 - protein, 97 aa, Artificial Sequence
  sequence from a gamma immunoglobulin heavy chain
STKGPSVFPLAPSSKSTSGGTAALGCLVKDYFPEPVTVSWNSGALTSGVHTFPAVLQSSGLYSLSSVVTVPSSSLGTQTYICNVNHKPSNTKVDKRV

SEQ ID NO: 3 - protein, 20 aa, Artificial Sequence
  spacer, human IgG1 hinge
AEPKSPDKTHTCPPCPKDPK

SEQ ID NO: 4 - protein, 15 aa, Artificial Sequence
  spacer, hinge spacer
EPKSCDKTHTCPPCP

SEQ ID NO: 5 - protein, 124 aa, Artificial Sequence
  anti-BCMA (B cell maturation target) Ab1 VH (heavy chain variable region)
QIQLVQSGPELVKPGSSVKLSCKTSGFTFSDSYMSWLKQVPGQSIEWIGNIYAGDGATHYHQKFKGKATLTVDTSSSTAYMDLSSLTSEDSALYFCARPLYTTAYYYVGGFAYWGQGTLVTVSS

SEQ ID NO: 6 - protein, 113 aa, Artificial Sequence
  anti-BCMA Ab1 VL (light chain variable region)
DIVMTQSPSSLAVSAGETVTINCKSSQSLLSSGNQKNYLAWYQQKPGQSPKLLIYWASTRQSGVPDRFIGSGSGTDFTLTISSVQAEDLAIYYCQQYYDTPLTFGSGTKLEIK

SEQ ID NO: 7 - protein, 121 aa, Artificial Sequence
  anti-BCMA Ab2 VH
EVKLVESGGGLVQPGRSLKLSCTASGFTFSNYDMAWVRQAPTKGLEWVASISTSGDTIYYRDSVKGRFTVSRDKAKSTLYLQMDSLRSEDTATYYCARHDYYDGYQSFAYWGQGTLVTVSS

SEQ ID NO: 8 - protein, 107 aa, Artificial Sequence
  anti-BCMA Ab2 VL
NTVMTQSPTSMSISVGDRVTMNCKASQNVGNNIAWYQQKPGQSPKLLIYYASNRYTGVPDRFTGSGSGTDFTLTINSVQAEDAAFYYCQRIYNSALTFGSGTKLEIK

SEQ ID NO: 9 - protein, 120 aa, Artificial Sequence
  anti-BCMA Ab3 VH
QVQLQQSGAALVKPGASVKMSCKASGYTFTDYWVSWVKQSHGKSLEWIGEIYPNSGPTNFNKKFKGKATLTVDKSTSTAYMELSRLTSEDSAIYYCTPRTVAPYNWFAYWGQGTLVTVSS

SEQ ID NO: 10 - protein, 106 aa, Artificial Sequence
  anti-BCMA Ab3 VL
DIVLTQSPALAVSPGERVSISCRASESVSTRMHWYQQKPGQQPKLLIYGASNLESGVPARFSGSGSGTDFTLTIDPVEADDTATYFCQQSWNDPYTFGAGTKLELK

SEQ ID NO: 11 - protein, 121 aa, Artificial Sequence
  anti-BCMA Ab4 VH
EVQLVESGGGLVQPGRSLKLSCSASGFIFSNFDMAWVRQAPRKGLEWVASITTSGGDTHYRDSVKGRFTVSRHNAKSTLYLQMDSLRSEDTATYYCARHVYYGLFWFFDFWGPGTMVTVSS

SEQ ID NO: 12 - protein, 108 aa, Artificial Sequence
  anti-BCMA Ab4 VL
NTVMTQSPKSIFISVGDRVTVNCKASQNVGTNVDWYQQKTGQSPKLLIYGASNRYTGVPDRFTGSGSGTDFTFTISNMQAEDLAVYYCMQSNTNPFTFGAGTKLELKR

SEQ ID NO: 13 - protein, 121 aa, Artificial Sequence
  anti-BCMA Ab5 VH
EVQLVESGGGLVQPGRSLKLSCTASGFTFSNYDMAWVRQAPTKGLEWVASISTSGDTIYYRDSVKGRFTVSRDKAKSTLYLQMDSLRSEDTATYYCARHDYYDGYQSFAYWGQGTLVTVSS

SEQ ID NO: 14 - protein, 108 aa, Artificial Sequence
  anti-BCMA Ab5 VL
DIVMTQSPSTLPASLGERVTISCRASQSISNYLNWYQQKPDGTIKPLIYYTSNLQSGVPSRFSGSGSGTDYSLTISSLEPEDFAMYYCQQDASFPWTFGGGTKLELKR

SEQ ID NO: 15 - protein, 119 aa, Artificial Sequence
  anti-BCMA Ab6 VH
EVQLQESGPGLVKPSQSLSLTCSVTGYPITNNYDWSWIRQFPGNKMEWMGYISDSGNTNYNPSLKSRISITRDTSKNQFFLQLNSVTTEDTATYYCASGYISYIPFAFWGQGTLVTVSS

SEQ ID NO: 16 - protein, 111 aa, Artificial Sequence
  anti-BCMA Ab6 VL
DIVLTQSPALAVSLGQRATISCRASQSVSISSYNLMQWYQQKPGQQPKLLIYDASNLASGIPARFSGSGSGTDFTLTIDPVQADDIATYYCQQSKDDPNTFGAGTKLEIKR

SEQ ID NO: 17 - protein, 119 aa, Artificial Sequence
  anti-BCMA Ab7 VH
EVQLQESGPGLVQPSQTLSLTCSVTGYPITNNYDWSWIRKFPGNKMEWMGYISDSGSTNYNPSLKSRISITRDTSKNQFFLQLNSVTTEDTATYYCASGYISYIPFGFWGQGTLVTVSS

SEQ ID NO: 18 - protein, 106 aa, Artificial Sequence
  anti-BCMA Ab7 VL
DIVLTQSPALAVSPGERVTISCRASESVSTRMHWYQQKPGQQPKLLIYGASNLESGVPARFSGSGSGTDFTLTIDPVEADDTATYFCQQSWNDPPTFGSGTKLEIK

SEQ ID NO: 19 - protein, 121 aa, Artificial Sequence; identical to SEQ ID NO: 13
  anti-BCMA Ab8 VH

SEQ ID NO: 20 - protein, 113 aa, Artificial Sequence
  anti-BCMA Ab8 VL
DIVMTQSPASQAVSAGEKVTMSCKSSQSLLYSGDQKNYLAWYQQKPGQSPKLLIYLASTRESGVPDRFIGSGSGTDFTLTISSVQAEDLADYYCQQHYSYPLTFGSGTKLEIK

SEQ ID NO: 21 - protein, 121 aa, Artificial Sequence
  anti-BCMA Ab9 VH
EVQLVESGGGLVQPGRSLKLSCAASGFTFSNYDMAWVRQAPTKGLEWVASISTSGDTIYYRDSVKGRFTVSRDNAKSTLYLQMDSLRSEDTATYYCTRHGYYDGYQSFDYWGQGTLVTVSS

SEQ ID NO: 22 - protein, 107 aa, Artificial Sequence
  anti-BCMA Ab9 VL
NTVMTQSPKSMSISVGDRVTMNCKASQNVGNNIAWYQQKPGQSPKLLIYYASNRYTGVPDRFTGGGYGTDFTLTINSVQAEDAATYYCQQWNYPSITFGSGTKLEIK

SEQ ID NO: 23 - protein, 122 aa, Artificial Sequence
  anti-BCMA Ab10 VH
EVQLVESGGGLVQPGRSMKLSCAASGFTFSNYDMAWVRQAPTKGLEWVASISPSGGSTYYRDSVKGRFTVSRDNAKSSLYLQMDSLRSEDTATYYCTRGDYGYNYAYWFAYWGQGTLVTVSS

SEQ ID NO: 24 - protein, 107 aa, Artificial Sequence
  anti-BCMA Ab10 VL
DIVMTQAPSSMPASLGERVTISCRASQGISNYLNWYQQKPDGTIKPLIYYTSNLQSGVPSRFSGSGSGTDYSLTISSLEPEDFAMYYCQQYDSSPLTFGAGTKLELK

SEQ ID NO: 25 - protein, 121 aa, Artificial Sequence
  anti-BCMA Ab11 VH
EVQLVESGGGLVQPGRSLKLSCEASGFTFSNYDMAWVRQAPTKGLEWVASISTSGDSIYYRDSVKGRFTVSRDNVKSTLYLQMDSLRSEDTATYYCARHGYYDGYQSFDYWGQGTLVTVSS

SEQ ID NO: 26 - protein, 107 aa, Artificial Sequence
  anti-BCMA Ab12 VL
DIVMTQSPSSLPASLGERVTISCRASQGISNNLNWYQQKPDGTIKPLIYYTSNLQSGVPSRFSGSGSGTDYSLTISSLEPEDFATYYCQQDETFPYTFGAGTKLELK

SEQ ID NO: 27 - protein, 121 aa, Artificial Sequence
  anti-BCMA Ab13 VH
EVQLVESGGGLVQPGRSLKLSCAASGFTFSNYDMAWVRQAPTKGLEWVASISPSGGSTYYRDSVKGRFTISRDNAKSTLYLQMDSLRSEDTATYYCATHNYYDGSSLFAYWGQGTLVTVSS

SEQ ID NO: 28 - protein, 106 aa, Artificial Sequence
  anti-BCMA Ab13 VL
DIVLTQSPALAVSPGERVTISCGANETVSTLVHWYQQKPGQQPKLLIYLASHLESGVPARFSGSGSGTDFTLTIDPVEADDTATYYCQQSWNDPPTFGGGTKLELK

SEQ ID NO: 29 - protein, 115 aa, Artificial Sequence
  anti-BCMA Ab14 VH
EVQLVESGGGLVQPGRSLKLSCAASGFIFSDYNMAWVRQAPKKGLEWVATIIYDGSSTNHGDSVKGRFTISRDNAKSTLYLQMDSLRSEDTATYYCATRPGPFAYWGQGTLVTVS

SEQ ID NO: 30 - protein, 111 aa, Artificial Sequence
  anti-BCMA Ab15 VL
DVVLTQTPPTLSATIGQSVSISCRSSQSLLHSNGNTYLHWLLQRPGQSPQFLIYLVSGLGSGVPNRFSGSGSGTDFTLKISGVEAEDLGIYYCVHGTHAWTVGGGTKLELK

SEQ ID NO: 31 - protein, 247 aa, Artificial Sequence
  transmembrane activator and calcium modulator and cyclophilin ligand (CAML) interactor (TACI) binder, 2H6 ScFv
EVQLQQSGPELVKPGASVRMSCKASGYTFTNYVMHWVKQKPGQGLEWIGYINPSNDDTKYTEKFKGKATLTSDKSSSTAYMELSSLTSEDSAVYYCARGTHGDYYALDYWGQGTSVTVSSGGGGAGGGGSGGGGSDIVLTQSPASLAVSLGQSVTISCRASESVEYYGTSLMQWYQQKPGQAPKLLIYGASNVESGVPARFSGSGSGTDFSLNIHPVEEDDIAMYFCQQSRKVPWTFGGGTKLEIKR

SEQ ID NO: 32 - protein, 5 aa, Artificial Sequence
  TACI binder 2H6, CDR H1
NYVMH

SEQ ID NO: 33 - protein, 17 aa, Artificial Sequence
  TACI binder 2H6, CDR H2
YINPSNDDTKYTEKFKG

SEQ ID NO: 34 - protein, 11 aa, Artificial Sequence
  TACI binder 2H6, CDR H3
GTHGDYYALDY

SEQ ID NO: 35 - protein, 15 aa, Artificial Sequence
  TACI binder 2H6, CDR L1
RASESVEYYGTSLMQ

SEQ ID NO: 36 - protein, 7 aa, Artificial Sequence
  TACI binder 2H6, CDR L2
GASNVES

SEQ ID NO: 37 - protein, 7 aa, Artificial Sequence
  TACI binder 2H6, CDR L3
QQSRKVP

SEQ ID NO: 38 - protein, 245 aa, Artificial Sequence
  TACI binder, 2G2 ScFv
QVTLKESGPGMLQPSQTLSLTCSFSGFSLSTFGMGVGWIRQPSGKGLEWLAHIWWDDAQYSNPALRSRLTISKDTSKNQVFLKIANVDTADTATYYCSRIHSYYSYDEGFAYWGQGTLVTVSSGGGGSGGGGSGGGGSDIVMTQSQKFMSTTVGDRVSITCKASQNVGTAVAWYQQKPGQSPKLLIYSASNRYTGVPDRFTGSGSGTDFTLTISNMQSEDLADYFCQQYSSYRTFGGGTKLEIKR

SEQ ID NO: 39 - protein, 7 aa, Artificial Sequence
  TACI binder 2G2, CDR H1
TFGMGVG

SEQ ID NO: 40 - protein, 16 aa, Artificial Sequence
  TACI binder 2G2, CDR H2
HIWWDDAQYSNPALRS

SEQ ID NO: 41 - protein, 14 aa, Artificial Sequence
  TACI binder 2G2, CDR H3
RIHSYYSYDEGFAY

SEQ ID NO: 42 - protein, 11 aa, Artificial Sequence
  TACI binder 2G2, CDR L1
KASQNVGTAVA

SEQ ID NO: 43 - protein, 7 aa, Artificial Sequence
  TACI binder 2G2, CDR L2
SASNRYT

SEQ ID NO: 44 - protein, 6 aa, Artificial Sequence
  TACI binder 2G2, CDR L3
QQYSSY

SEQ ID NO: 45 - protein, 115 aa, Artificial Sequence
  TACI binder, 1G6 VH
QVQLKQSGPGLVAPSQSLSITCTVSGFSLTSYGVDWVRQSPGKGLEWLGIIWGGGRTNYNSAFKSRLSISKDNSKSQVFLKMNSLQTDDTAMYYCASGDRAADYWGQGTSVTVSS

SEQ ID NO: 46 - protein, 107 aa, Artificial Sequence
  TACI binder ,1G6 VL
DIVMTQSQKFMSTTVGDRVTITCKASQNVGTAVAWYQQKPGQSPKLLIYSASNRYTGVPVRFTGSGSGTDFTLTINNMQSEDLADYFCQQYSSYPLTFGAGTKLELK

SEQ ID NO: 47 - protein, 5 aa, Artificial Sequence
  TACI binder 1G6, CDR H1
SYGVD

SEQ ID NO: 48 - protein, 16 aa, Artificial Sequence
  TACI binder 1G6, CDR H2
IIWGGGRTNYNSAFKS

SEQ ID NO: 49 - protein, 7 aa, Artificial Sequence
  TACI binder 1G6, CDR H3
GDRAADY

SEQ ID NO: 50 - protein, 11 aa, Artificial Sequence
  TACI binder 1G6, CDR L1
KASQNVGTAVA

SEQ ID NO: 51 - protein, 7 aa, Artificial Sequence
  TACI binder 1G6, CDR L2
SASNRYT

SEQ ID NO: 52 - protein, 7 aa, Artificial Sequence
  TACI binder 1G6, CDR L3
QQYSSYP

SEQ ID NO: 53 - protein, 114 aa, Artificial Sequence
  TACI binder, 4B11 VH
EVQLQQSVAELVRPGASVKLSCTASGFNIKNTYIHWVKQRPEQGLEWIGKIDPANGNSEYAPKFQGKATITADTSSNTAYLQLSSLTSEDTTIYYCTSGYGAYWGQGTTLTVSS

SEQ ID NO: 54 - protein, 111 aa, Artificial Sequence
  TACI binder, 4B11 VL
DIVLSQSPSSLAVSIGEKVTLSCKSSQSLLYSSNQKNYLAWFQQKPGQSLKLLIYWASTREFGVPDRFTGSGSGTDFTLTISSVKTEDLAVYYCQQYYTWTFGGGTKLEIK

SEQ ID NO: 55 - protein, 5 aa, Artificial Sequence
  TACI binder 4B11, CDR H1
NTYIH

SEQ ID NO: 56 - protein, 17 aa, Artificial Sequence
  TACI binder 4B11, CDR H2
KIDPANGNSEYAPKFQG

SEQ ID NO: 57 - protein, 5 aa, Artificial Sequence
  TACI binder 4B11, CDR H3
GYGAY

SEQ ID NO: 58 - protein, 17 aa, Artificial Sequence
  TACI binder 4B11, CDR L1
KSSQSLLYSSNQKNYLA

SEQ ID NO: 59 - protein, 7 aa, Artificial Sequence
  TACI binder 4B11, CDR L2
WASTREF

SEQ ID NO: 60 - protein, 6 aa, Artificial Sequence
  TACI binder 4B11, CDR L3
QQYYTW

SEQ ID NO: 61 - protein, 7 aa, Artificial Sequence
  CD19-binding domain VH CDR, CDR1
GYAFSSS

SEQ ID NO: 62 - protein, 6 aa, Artificial Sequence
  CD19-binding domain VH CDR, CDR2
YPGDED

SEQ ID NO: 63 - protein, 10 aa, Artificial Sequence
  CD19-binding domain VH CDR, CDR3
SLLYGDYLDY

SEQ ID NO: 64 - protein, 10 aa, Artificial Sequence
  CD19-binding domain VL CDR, CDR1
SASSSVSYMH

SEQ ID NO: 65 - protein, 7 aa, Artificial Sequence
  CD19-binding domain VL CDR, CDR2
DTSKLAS

SEQ ID NO: 66 - protein, 9 aa, Artificial Sequence
  CD19-binding domain VL CDR, CDR3
QQWNINPLT

SEQ ID NO: 67 - protein, 119 aa, Artificial Sequence
  VH sequence from murine monoclonal antibody
QVQLQQSGPELVKPGASVKISCKASGYAFSSSWMNWVKQRPGKGLEWIGRIYPGDEDTNYSGKFKDKATLTADKSSTTAYMQLSSLTSEDSAVYFCARSLLYGDYLDYWGQGTTLTVSS

SEQ ID NO: 68 - protein, 8 aa, Artificial Sequence
  VH CDR1
GFTFSDSY

SEQ ID NO: 69 - protein, 8 aa, Artificial Sequence
  VH CDR2
IYAGDGAT

SEQ ID NO: 70 - protein, 17 aa, Artificial Sequence
  VH CDR3
ARPLYTTAYYYVGGFAY

SEQ ID NO: 71 - protein, 12 aa, Artificial Sequence
  VL CDR1
QSLLSSGNQKNY

SEQ ID NO: 72 - protein, 3 aa, Artificial Sequence
  VL CDR2
WAS

SEQ ID NO: 73 - protein, 9 aa, Artificial Sequence
  VL CDR3
QQYYDTPLT

SEQ ID NO: 74 - protein, 6 aa, Artificial Sequence
  DXL motif of TACI cysteine-rich domain (CRD)
  MISC_FEATURE (1)..(1): Xaa may be Phe, Tyr or Trp
  misc_feature (3)..(3): Xaa can be any naturally occurring amino acid
  MISC_FEATURE (5)..(5): Xaa may be Val or Thr
  MISC_FEATURE (6)..(6): Xaa may be Arg or Gly
XDXLXX

SEQ ID NO: 75 - protein, 107 aa, Artificial Sequence
  VL sequence from murine monoclonal antibody
QIVLTQSPAIMSASPGEKVTMTCSASSSVSYMHWYQQKSGTSPKRWIYDTSKLASGVPDRFSGSGSGTSYFLTINNMEAEDAATYYCQQWNINPLTFGAGTKLELKR

SEQ ID NO: 76 - protein, 241 aa, Artificial Sequence
  VH-VL scFv sequence from murine monoclonal antibody
QVQLQQSGPELVKPGASVKISCKASGYAFSSSWMNWVKQRPGKGLEWIGRIYPGDEDTNYSGKFKDKATLTADKSSTTAYMQLSSLTSEDSAVYFCARSLLYGDYLDYWGQGTTLTVSSGGGGSGGGGSGGGGSQIVLTQSPAIMSASPGEKVTMTCSASSSVSYMHWYQQKSGTSPKRWIYDTSKLASGVPDRFSGSGSGTSYFLTINNMEAEDAATYYCQQWNINPLTFGAGTKLELKR

SEQ ID NO: 77 - protein, 20 aa, Artificial Sequence
  cleavage site, 2A-like sequence
RAEGRGSLLTCGDVEENPGP

SEQ ID NO: 78 - protein, 5 aa, Artificial Sequence
  glycine-serine linker
GGGGS

SEQ ID NO: 79 - protein, 8 aa, Artificial Sequence
  VH CDR1
GFIFSDYN

SEQ ID NO: 80 - protein, 8 aa, Artificial Sequence
  VH CDR2
IIYDGSST

SEQ ID NO: 81 - protein, 9 aa, Artificial Sequence
  VH CDR3
ATRPGPFAY

SEQ ID NO: 82 - protein, 11 aa, Artificial Sequence
  VL CDR1
QSLLHSNGNTY

SEQ ID NO: 83 - protein, 3 aa, Artificial Sequence
  VL CDR2
LVS

SEQ ID NO: 84 - protein, 8 aa, Artificial Sequence
  VL CDR3
VHGTHAWT

SEQ ID NO: 85 - protein, 6 aa, Artificial Sequence
  MMP-1, sequence cleavable with MMP enzyme
PLGLWA

SEQ ID NO: 86 - protein, 6 aa, Artificial Sequence
  MMP-2, sequence cleavable with MMP enzyme
PAGLAG

SEQ ID NO: 87 - protein, 6 aa, Artificial Sequence
  MMP-9, sequence cleavable with MMP enzyme
PLGLAG

SEQ ID NO: 88 - protein, 6 aa, Artificial Sequence
  scrambled MMP-9 cleavable linker (negative control)
LALGPG